European Patent Application EP 4 722 228 A1, published April 8, 2026. Title: ＭｕＳＫを標的とする新規化合物及びその用途. Applicant: 国立大学法人　東京大学. Application JP. The sequence listing filed with the application follows.

SEQUENCE LISTING (61 sequences)

SEQ ID NO: 1 - protein, 76 aa, Homo sapiens [sequence omitted]

SEQ ID NO: 2 - protein, 15 aa, synthetic construct
YPSYHTNVVASLKRC

SEQ ID NO: 3 - protein, 13 aa, synthetic construct
YFPTNVVSLLKSC

SEQ ID NO: 4 - protein, 17 aa, synthetic construct
YWYLQPGYVNIVTSYHC

SEQ ID NO: 5 - protein, 27 aa, synthetic construct
YLPEFSWPESFVLFLRQRQRQLGRGAE

SEQ ID NO: 6 - protein, 15 aa, synthetic construct
YLPEFSWPESFVLFL

SEQ ID NO: 7 - protein, 15 aa, synthetic construct
YSRYCEWIALNRWII

SEQ ID NO: 8 - protein, 16 aa, synthetic construct
YSAWQHLASWVAHSQN

SEQ ID NO: 9 - protein, 28 aa, synthetic construct
YAPCSLELHDWILVSLAAAAAAARTGGG

SEQ ID NO: 10 - protein, 16 aa, synthetic construct
YAPCSLELHDWILVSL

SEQ ID NO: 11 - protein, 14 aa, synthetic construct
YXSYHTNVVASLKR

SEQ ID NO: 12 - protein, 4 aa, synthetic construct
IQPR

SEQ ID NO: 13 - protein, 4 aa, synthetic construct
KPGV

SEQ ID NO: 14 - protein, 4 aa, synthetic construct
WDRG

SEQ ID NO: 15 - protein, 4 aa, synthetic construct
KPGT

SEQ ID NO: 16 - protein, 4 aa, synthetic construct
PFGV

SEQ ID NO: 17 - protein, 4 aa, synthetic construct
YFVG

SEQ ID NO: 18 - protein, 4 aa, synthetic construct
LEGM

SEQ ID NO: 19 - protein, 4 aa, synthetic construct
TGPQ

SEQ ID NO: 20 - protein, 4 aa, synthetic construct
WNTP

SEQ ID NO: 21 - protein, 4 aa, synthetic construct
IRPQ

SEQ ID NO: 22 - protein, 21 aa, synthetic construct
IQPRYPSYHTNVVASLKRIRY

SEQ ID NO: 23 - protein, 21 aa, synthetic construct
KPGVYPSYHTNVVASLKRMMP

SEQ ID NO: 24 - protein, 21 aa, synthetic construct
WDRGYPSYHTNVVASLKRQGI

SEQ ID NO: 25 - protein, 21 aa, synthetic construct
KPGTYPSYHTNVVASLKRFMP

SEQ ID NO: 26 - protein, 22 aa, synthetic construct
PFGVYPSYHTNVVASLKRTGPQ

SEQ ID NO: 27 - protein, 22 aa, synthetic construct
YFVGYPSYHTNVVASLKRWNTP

SEQ ID NO: 28 - protein, 22 aa, synthetic construct
LEGMYLSYHTNVVASLKRIRPQ

SEQ ID NO: 29 - protein, 22 aa, synthetic construct
LEGMYPSYHTNVVASLKRIRPQ

SEQ ID NO: 30 - protein, 4 aa, synthetic construct
TNVV

SEQ ID NO: 31 - protein, 4 aa, synthetic construct
TNIV

SEQ ID NO: 32 - protein, 4 aa, synthetic construct
VNVV

SEQ ID NO: 33 - protein, 4 aa, synthetic construct
VNIV

SEQ ID NO: 34 - protein, 734 aa, synthetic construct
MDSKGSSQKGSRLLLLLVVSNLLLCQGVVSGSLPKAPVITTPLETVDALVEEVATFMCAVESYPQPEISWTRNKILIKLFDTRYSIRENGQLLTILSVEDSDDGIYCCIANNGVGGAVESCGALQVKMKPKITRPPINVKIIEGLKAVLPCTTMGNPKPSVSWIKGDNALRENSRIAVLESGSLRIHNVQKEDAGQYRCVAKNSLGTAYSKLVKLEVEVFARILRAPESHNVTFGSFVTLRCTAIGIPVPTISWIENGNAVSSGSIQESVKDRVIDSRLQLFITKPGLYTCIATNKHGEKFSTAKAAATVSIAEWSKSQKDSQGYCAQYRGEVCDAVLAKDALVFFNTSYRDPEDAQELLIHTAWNELKAVSPLCRPAAEALLCNHLFQECSPGVVPTPMPICREYCLAVKELFCAKEWQAMEGKAHRGLYRSGMHLLPVPECSKLPSMHRDPTACTRLPYLDYKKENITTFPSITSSRPSADIPNLPASTSSFAVSPAYSMTVESRDKTHTCPPCPAPELLGGPSVFLFPPKPKDTLMISRTPEVTCVVVDVSHEDPEVKFNWYVDGVEVHNAKTKPREEQYNSTYRVVSVLTVLHQDWLNGKEYKCKVSNKALPAPIEKTISKAKGQPREPQVYTLPPSRDELTKNQVSLTCLVKGFYPSDIAVEWESNGQPENNYKTTPPVLDSDGSFFLYSKLTVDKSRWQQGNVFSCSVMHEALHNHYTQKSLSLSPGK

SEQ ID NO: 35 - protein, 15 aa, synthetic construct
YRQFNRRTHEVWNLD

SEQ ID NO: 36 - protein, 14 aa, synthetic construct
YWYYAWDQTYKAFP

SEQ ID NO: 37 - protein, 14 aa, synthetic construct
YPSYHTNVVASLKR

SEQ ID NO: 38 - protein, 93 aa, synthetic construct
MQIFVKIQPRYPSYHTNVVASLKRIRYKTITLEVEPSDTIENVKAKIQDKEGIPPDQQRLIFAGKQLEDGRTLSDYNIQKESTLHLVLRLRGG

SEQ ID NO: 39 - protein, 93 aa, synthetic construct
MQIFVKKPGVYPSYHTNVVASLKRMMPKTITLEVEPSDTIENVKAKIQDKEGIPPDQQRLIFAGKQLEDGRTLSDYNIQKESTLHLVLRLRGG

SEQ ID NO: 40 - protein, 93 aa, synthetic construct
MQIFVKWDRGYPSYHTNVVASLKRQGIKTITLEVEPSDTIENVKAKIQDKEGIPPDQQRLIFAGKQLEDGRTLSDYNIQKESTLHLVLRLRGG

SEQ ID NO: 41 - protein, 93 aa, synthetic construct
MQIFVKKPGTYPSYHTNVVASLKRFMPKTITLEVEPSDTIENVKAKIQDKEGIPPDQQRLIFAGKQLEDGRTLSDYNIQKESTLHLVLRLRGG

SEQ ID NO: 42 - protein, 94 aa, synthetic construct
MQIFVKPFGVYPSYHTNVVASLKRTGPQKTITLEVEPSDTIENVKAKIQDKEGIPPDQQRLIFAGKQLEDGRTLSDYNIQKESTLHLVLRLRGG

SEQ ID NO: 43 - protein, 94 aa, synthetic construct
MQIFVKYFVGYPSYHTNVVASLKRWNTPKTITLEVEPSDTIENVKAKIQDKEGIPPDQQRLIFAGKQLEDGRTLSDYNIQKESTLHLVLRLRGG

SEQ ID NO: 44 - protein, 94 aa, synthetic construct
MQIFVKLEGMYLSYHTNVVASLKRIRPQKTITLEVEPSDTIENVKAKIQDKEGIPPDQQRLIFAGKQLEDGRTLSDYNIQKESTLHLVLRLRGG

SEQ ID NO: 45 - protein, 94 aa, synthetic construct
MQIFVKLEGMYPSYHTNVVASLKRIRPQKTITLEVEPSDTIENVKAKIQDKEGIPPDQQRLIFAGKQLEDGRTLSDYNIQKESTLHLVLRLRGG

SEQ ID NO: 46 - DNA, 300 bp, synthetic construct
  source 1..300: mol_type = other DNA
atgcatcaccaccaccaccacatgcagatcttcgtcaagattcagccgaggtatccttcgtatcatactaatgttgtggcgagtctgaagcgtattcggtataaaaccataactctagaagtggaaccgagcgataccatcgaaaacgtgaaagcgaaaatccaggataaagaaggcatcccgccggatcagcagcgtctgatctttgcgggcaaacagctggaagatggccgcaccctgtctgattataacatccagaaagagtcgaccctgcatctggtcttaagactgcgtgggggc

SEQ ID NO: 47 - DNA, 300 bp, synthetic construct
  source 1..300: mol_type = other DNA
atgcatcaccaccaccaccacatgcagatcttcgtcaagaagccgggggtttatccttcgtatcatactaatgttgtggcgagtctgaagcgtatgatgccgaaaaccataactctagaagtggaaccgagcgataccatcgaaaacgtgaaagcgaaaatccaggataaagaaggcatcccgccggatcagcagcgtctgatctttgcgggcaaacagctggaagatggccgcaccctgtctgattataacatccagaaagagtcgaccctgcatctggtcttaagactgcgtgggggc

SEQ ID NO: 48 - DNA, 300 bp, synthetic construct
  source 1..300: mol_type = other DNA
atgcatcaccaccaccaccacatgcagatcttcgtcaagtgggatcgtgggtatccttcgtatcatactaatgttgtggcgagtctgaagcgtcagggtattaaaaccataactctagaagtggaaccgagcgataccatcgaaaacgtgaaagcgaaaatccaggataaagaaggcatcccgccggatcagcagcgtctgatctttgcgggcaaacagctggaagatggccgcaccctgtctgattataacatccagaaagagtcgaccctgcatctggtcttaagactgcgtgggggc

SEQ ID NO: 49 - DNA, 300 bp, synthetic construct
  source 1..300: mol_type = other DNA
atgcatcaccaccaccaccacatgcagatcttcgtcaagaagccggggacgtatccttcgtatcatactaatgttgtggcgagtctgaagcgttttatgcctaaaaccataactctagaagtggaaccgagcgataccatcgaaaacgtgaaagcgaaaatccaggataaagaaggcatcccgccggatcagcagcgtctgatctttgcgggcaaacagctggaagatggccgcaccctgtctgattataacatccagaaagagtcgaccctgcatctggtcttaagactgcgtgggggc

SEQ ID NO: 50 - DNA, 303 bp, synthetic construct
  source 1..303: mol_type = other DNA
atgcatcaccaccaccaccacatgcagatcttcgtcaagccgtttggggtgtatccttcgtatcatactaatgttgtggcgagtctgaagcgtactggtcctcagaaaaccataactctagaagtggaaccgagcgataccatcgaaaacgtgaaagcgaaaatccaggataaagaaggcatcccgccggatcagcagcgtctgatctttgcgggcaaacagctggaagatggccgcaccctgtctgattataacatccagaaagagtcgaccctgcatctggtcttaagactgcgtgggggc

SEQ ID NO: 51 - DNA, 303 bp, synthetic construct
  source 1..303: mol_type = other DNA
atgcatcaccaccaccaccacatgcagatcttcgtcaagtattttgttgggtatccttcgtatcatactaatgttgtggcgagtctgaagcgttggaatacgccgaaaaccataactctagaagtggaaccgagcgataccatcgaaaacgtgaaagcgaaaatccaggataaagaaggcatcccgccggatcagcagcgtctgatctttgcgggcaaacagctggaagatggccgcaccctgtctgattataacatccagaaagagtcgaccctgcatctggtcttaagactgcgtgggggc

SEQ ID NO: 52 - DNA, 303 bp, synthetic construct
  source 1..303: mol_type = other DNA
atgcatcaccaccaccaccacatgcagatcttcgtcaagttggagggtatgtatctttcgtatcatactaatgttgtggcgagtctgaagcgtattaggccgcagaaaaccataactctagaagtggaaccgagcgataccatcgaaaacgtgaaagcgaaaatccaggataaagaaggcatcccgccggatcagcagcgtctgatctttgcgggcaaacagctggaagatggccgcaccctgtctgattataacatccagaaagagtcgaccctgcatctggtcttaagactgcgtgggggc

SEQ ID NO: 53 - DNA, 303 bp, synthetic construct
  source 1..303: mol_type = other DNA
atgcatcaccaccaccaccacatgcagatcttcgtcaagttggagggtatgtatccttcgtatcatactaatgttgtggcgagtctgaagcgtattaggccgcagaaaaccataactctagaagtggaaccgagcgataccatcgaaaacgtgaaagcgaaaatccaggataaagaaggcatcccgccggatcagcagcgtctgatctttgcgggcaaacagctggaagatggccgcaccctgtctgattataacatccagaaagagtcgaccctgcatctggtcttaagactgcgtgggggc

SEQ ID NO: 54 - protein, 205 aa, synthetic construct
MQIFVKLEGMYLSYHTNVVASLKRIRPQKTITLEVEPSDTIENVKAKIQDKEGIPPDQQRLIFAGKQLEDGRTLSDYNIQKESTLHLVLRLRGGAPAPAPAPAPAPAPATSMQIFVKLEGMYLSYHTNVVASLKRIRPQKTITLEVEPSDTIENVKAKIQDKEGIPPDQQRLIFAGKQLEDGRTLSDYNIQKESTLHLVLRLRGG

SEQ ID NO: 55 - DNA, 648 bp, synthetic construct
  source 1..648: mol_type = other DNA
atgcatcaccaccaccaccacgctagcatgcagatcttcgtcaagttggagggtatgtatctttcgtatcatactaatgttgtggcgagtctgaagcgtattaggccgcagaaaaccataactctagaagtggaaccgagcgataccatcgaaaacgtgaaagcgaaaatccaggataaagaaggcatcccgccggatcagcagcgtctgatctttgcgggcaaacagctggaagatggccgcaccctgtctgattataacatccagaaagagtcgaccctgcatctggtcttaagactgcgtgggggcgctccagcacctgctcccgctccagcacctgccccagcacctgccactagcatgcagatcttcgtcaagttggagggtatgtatctttcgtatcatactaatgttgtggcgagtctgaagcgtattaggccgcagaaaaccataactctagaagtggaaccgagcgataccatcgaaaacgtgaaagcgaaaatccaggataaagaaggcatcccgccggatcagcagcgtctgatctttgcgggcaaacagctggaagatggccgcaccctgtctgattataacatccagaaagagtcgaccctgcatctggtcttaagactgcgtgggggcactagt

SEQ ID NO: 56 - protein, 427 aa, synthetic construct
MQIFVKLEGMYLSYHTNVVASLKRIRPQKTITLEVEPSDTIENVKAKIQDKEGIPPDQQRLIFAGKQLEDGRTLSDYNIQKESTLHLVLRLRGGAPAPAPAPAPAPAPATSMQIFVKLEGMYLSYHTNVVASLKRIRPQKTITLEVEPSDTIENVKAKIQDKEGIPPDQQRLIFAGKQLEDGRTLSDYNIQKESTLHLVLRLRGGAPAPAPAPAPAPAPATSMQIFVKLEGMYLSYHTNVVASLKRIRPQKTITLEVEPSDTIENVKAKIQDKEGIPPDQQRLIFAGKQLEDGRTLSDYNIQKESTLHLVLRLRGGAPAPAPAPAPAPAPATSMQIFVKLEGMYLSYHTNVVASLKRIRPQKTITLEVEPSDTIENVKAKIQDKEGIPPDQQRLIFAGKQLEDGRTLSDYNIQKESTLHLVLRLRGG

SEQ ID NO: 57 - DNA, 1314 bp, synthetic construct
  source 1..1314: mol_type = other DNA
atgcatcaccaccaccaccacgctagcatgcagatcttcgtcaagttggagggtatgtatctttcgtatcatactaatgttgtggcgagtctgaagcgtattaggccgcagaaaaccataactctagaagtggaaccgagcgataccatcgaaaacgtgaaagcgaaaatccaggataaagaaggcatcccgccggatcagcagcgtctgatctttgcgggcaaacagctggaagatggccgcaccctgtctgattataacatccagaaagagtcgaccctgcatctggtcttaagactgcgtgggggcgctccagcacctgctcccgctccagcacctgccccagcacctgccactagcatgcagatcttcgtcaagttggagggtatgtatctttcgtatcatactaatgttgtggcgagtctgaagcgtattaggccgcagaaaaccataactctagaagtggaaccgagcgataccatcgaaaacgtgaaagcgaaaatccaggataaagaaggcatcccgccggatcagcagcgtctgatctttgcgggcaaacagctggaagatggccgcaccctgtctgattataacatccagaaagagtcgaccctgcatctggtcttaagactgcgtgggggcgctccagcacctgctcccgctccagcacctgccccagcacctgccactagcatgcagatcttcgtcaagttggagggtatgtatctttcgtatcatactaatgttgtggcgagtctgaagcgtattaggccgcagaaaaccataactctagaagtggaaccgagcgataccatcgaaaacgtgaaagcgaaaatccaggataaagaaggcatcccgccggatcagcagcgtctgatctttgcgggcaaacagctggaagatggccgcaccctgtctgattataacatccagaaagagtcgaccctgcatctggtcttaagactgcgtgggggcgctccagcacctgctcccgctccagcacctgccccagcacctgccactagcatgcagatcttcgtcaagttggagggtatgtatctttcgtatcatactaatgttgtggcgagtctgaagcgtattaggccgcagaaaaccataactctagaagtggaaccgagcgataccatcgaaaacgtgaaagcgaaaatccaggataaagaaggcatcccgccggatcagcagcgtctgatctttgcgggcaaacagctggaagatggccgcaccctgtctgattataacatccagaaagagtcgaccctgcatctggtcttaagactgcgtgggggcactagt

SEQ ID NO: 58 - protein, 169 aa, synthetic construct
MQIFVKTLTGKTITLEVEPSDTIENVKAKIQDKEGIPPDQQRLIFAGKQLEDGRTLSDYNIQKESTLHLVLRLRGGAPAPAPAPAPAPAPATSMQIFVKTLTGKTITLEVEPSDTIENVKAKIQDKEGIPPDQQRLIFAGKQLEDGRTLSDYNIQKESTLHLVLRLRGG

SEQ ID NO: 59 - DNA, 543 bp, synthetic construct
  source 1..543: mol_type = other DNA
atgcatcaccaccaccaccacgctagcatgcagatcttcgtcaagacgttaaccggtaaaaccataactctagaagtggaaccgagcgataccatcgaaaacgtgaaagcgaaaatccaggataaagaaggcatcccgccggatcagcagcgtctgatctttgcgggcaaacagctggaagatggccgcaccctgtctgattataacatccagaaagagtcgaccctgcatctggtcttaagactgcgtgggggcgctccagcacctgctcccgctccagcacctgccccagcacctgccactagcatgcagatcttcgtcaagacgttaaccggtaaaaccataactctagaagtggaaccgagcgataccatcgaaaacgtgaaagcgaaaatccaggataaagaaggcatcccgccggatcagcagcgtctgatctttgcgggcaaacagctggaagatggccgcaccctgtctgattataacatccagaaagagtcgaccctgcatctggtcttaagactgcgtgggggcactagttaa

SEQ ID NO: 60 - protein, 421 aa, synthetic construct
MQIFVKLEGMYLSYHTNVVASLKRIRPQKTITLEVEPSDTIENVKAKIQDKEGIPPDQQRLIFAGKQLEDGRTLSDYNIQKESTLHLVLRLRGGEAAAKEAAAKEAAAKMQIFVKLEGMYLSYHTNVVASLKRIRPQKTITLEVEPSDTIENVKAKIQDKEGIPPDQQRLIFAGKQLEDGRTLSDYNIQKESTLHLVLRLRGGEAAAKEAAAKEAAAKMQIFVKLEGMYLSYHTNVVASLKRIRPQKTITLEVEPSDTIENVKAKIQDKEGIPPDQQRLIFAGKQLEDGRTLSDYNIQKESTLHLVLRLRGGEAAAKEAAAKEAAAKMQIFVKLEGMYLSYHTNVVASLKRIRPQKTITLEVEPSDTIENVKAKIQDKEGIPPDQQRLIFAGKQLEDGRTLSDYNIQKESTLHLVLRLRGG

SEQ ID NO: 61 - protein, 413 aa, synthetic construct
MQIFVKLEGMYLSYHTNVVASLKRIRPQKTITLEVEPSDTIENVKAKIQDKEGIPPDQQRLIFAGKQLEDGRTLSDYNIQKESTLHLVLRLREAAAKEAAAKEAAAKMQIFVKLEGMYLSYHTNVVASLKRIRPQKTITLEVEPSDTIENVKAKIQDKEGIPPDQQRLIFAGKQLEDGRTLSDYNIQKESTLHLVLRLREAAAKEAAAKEAAAKMQIFVKLEGMYLSYHTNVVASLKRIRPQKTITLEVEPSDTIENVKAKIQDKEGIPPDQQRLIFAGKQLEDGRTLSDYNIQKESTLHLVLRLREAAAKEAAAKEAAAKMQIFVKLEGMYLSYHTNVVASLKRIRPQKTITLEVEPSDTIENVKAKIQDKEGIPPDQQRLIFAGKQLEDGRTLSDYNIQKESTLHLVLRLR